European Patent Application EP 4 488 364 A1, published January 8, 2025. Title: Hypoimmune Stem Cell, Hypoimmune Cell Differentiated or Derived From Stem Cell and Preparation Method Thereof. Applicant: 주식회사 툴젠. Application KR PCT230301, filed March 6, 2023. The sequence listing filed with the application follows.

SEQUENCE LISTING (27 sequences)

SEQ ID NO: 1 - RNA, 20 nt, synthetic construct
  source 1..20: mol_type = other RNA
gtcaccaatcctgtccctag

SEQ ID NO: 2 - DNA, 20 bp, synthetic construct
  source 1..20: mol_type = other DNA
attccccttcgacctactct

SEQ ID NO: 3 - DNA, 21 bp, synthetic construct
  source 1..21: mol_type = other DNA
ccgtaaatactccacccattg

SEQ ID NO: 4 - DNA, 20 bp, synthetic construct
  source 1..20: mol_type = other DNA
ctgaagcaaacatggacagg

SEQ ID NO: 5 - DNA, 20 bp, synthetic construct
  source 1..20: mol_type = other DNA
gataccccgaagagtgagtt

SEQ ID NO: 6 - DNA, 20 bp, synthetic construct
  source 1..20: mol_type = other DNA
gcctttcatcaccaccattc

SEQ ID NO: 7 - DNA, 21 bp, synthetic construct
  source 1..21: mol_type = other DNA
agtctccgacctcctccttca

SEQ ID NO: 8 - DNA, 21 bp, synthetic construct
  source 1..21: mol_type = other DNA
tctctctcagcttcagccact

SEQ ID NO: 9 - DNA, 20 bp, synthetic construct
  source 1..20: mol_type = other DNA
cccacctttagcaccacttt

SEQ ID NO: 10 - DNA, 1446 bp, Synthetic construct
  source 1..1446: mol_type = other DNA
attccccttcgacctactctcttccgcattggagtcgctttaactggccctggctttggcagcctgtgctgacccatgcagtcctccttaccatccctccctcgacttcccctcttccgatgttgagcccctccagccggtcctggactttgtctccttccctgccctgccctctcctgaacctgagccagctcccatagctcagtctggtctatctgcctggccctggccattgtcactttgcgctgccctcctctcgcccccgagtgcccttgctgtgccgccggaactctgccctctaacgctgccgtctctctcctgagtccggaccactttgagctctactggcttctgcgccgcctctggcccactgtttccccttcccaggcaggtcctgctttctctgacctgcattctctcccctgggcctgtgccgctttctgtctgcagcttgtggcctgggtcacctctacggctggcccagatccttccctgccgcctccttcaggttccgtcttcctccactccctcttccccttgctctctgctgtgttgctgcccaaggatgctctttccggagcacttccttctcggcgctgcaccacgtgatgtcctctgagcggatcctccccgtgtctgggtcctctccgggcatctctcctccctcacccaaccccatgccgtcttcactcgctgggttcccttttccttctccttctggggcctgtgccatctctcgtttcttaggatggccttctccgacggatgtctcccttgcgtcccgcctccccttcttgtaggcctgcatcatcaccgtttttctggacaaccccaaagtaccccgtctccctggctttagccacctctccatcctcttgctttctttgcctggacaccccgttctcctgtggattcgggtcacctctcactcctttcatttgggcagctcccctaccccccttacctctctagtctgtgctagctcttccagccccctgtcatggcatcttccaggggtccgagagctcagctagtcttcttcctccaacccgggcccctatgtccacttcaggacagcatgtttgctgcctccagggatcctgtgtccccgagctgggaccaccttatattcccagggccggttaatgtggctctggttctgggtacttttatctgtcccctccaccccacagtggggccactacaagtttgtacaaaaaagcaggctgtcgacattgattattgactagttattaatagtaatcaattacggggtcattagttcatagcccatatatggagttccgcgttacataacttacggtaaatggcccgcctggctgaccgcccaacgacccccgcccattgacgtcaataatgacgtatgttcccatagtaacgccaatagggactttccattgacgtcaatgggtggagtatttacgg

SEQ ID NO: 11 - DNA, 1790 bp, synthetic construct
  source 1..1790: mol_type = other DNA
ctgaagcaaacatggacagggcgctggacgatgaaagatggccttcataaaatgcaaagtgaacacgtttcactctcatgtcaacctgtaaatgattatttttcaccaaaccaagacttcaaagttacttggtccagaatgaaaagtgggactttctctgtcctggcttactatctgagctcctcacaaaatacaattatcaatgaatcccgattctcatggaacaaagagctgataaaccagagtgacttctctatgaatttgatggatcttaatctttcagacagtggggaatatttatgcaatatttcttcggatgaatatactttacttaccatccacacagtgcatgtagaaccgagccaagaaacagcttcccataacaaaggcttatggattttggtgccctctgcgattttggcagcttttctgctgatttggagcgtaaaatgttgcagagcccagctagaagccaggaggagcagacaccctgctgatggagcccaacaagaaagatgttgtgtccctcctggtgagcgctgtcccagtgcacccgataatggcgaagaaaatgtgcctctttcaggaaaagtatagaacttgtttattgcagcttataatggttacaaataaagcaatagcatcacaaatttcacaaataaagcatttttttcactgcattctagttgtggtttgtccaaactcatcaatgtatcttagtcgacagtactaagcttacccagctttcttgtacaaagtgggggacaggattggtgacagaaaagccccatccttaggcctcctccttcctagtctcctgatattgggtctaacccccacctcctgttaggcagattccttatctggtgacacacccccatttcctggagccatctctctccttgccagaacctctaaggtttgcttacgatggagccagagaggatcctgggagggagagcttggcagggggtgggagggaagggggggatgcgtgacctgcccggttctcagtggccaccctgcgctaccctctcccagaacctgagctgctctgacgcggccgtctggtgcgtttcactgatcctggtgctgcagcttccttacacttcccaagaggagaagcagtttggaaaaacaaaatcagaataagttggtcctgagttctaactttggctcttcacctttctagtccccaatttatattgttcctccgtgcgtcagttttacctgtgagataaggccagtagccagccccgtcctggcagggctgtggtgaggaggggggtgtccgtgtggaaaactccctttgtgagaatggtgcgtcctaggtgttcaccaggtcgtggccgcctctactccctttctctttctccatccttctttccttaaagagtccccagtgctatctgggacatattcctccgcccagagcagggtcccgcttccctaaggccctgctctgggcttctgggtttgagtccttggcaagcccaggagaggcgctcaggcttccctgtcccccttcctcgtccaccatctcatgcccctggctctcctgccccttccctacaggggttcctggctctgctcttcagactgagccccgttcccctgcatccccgttcccctgcatcccccttcccctgcatcccccagaggccccaggccacctacttggcctggaccccacgagaggccaccccagccctgtctaccaggctgccttttgggtggattctcctccaactgtggggtgactgcttggcaaactcactcttcggggtatc

SEQ ID NO: 12 - DNA, 725 bp, synthetic construct
  source 1..725: mol_type = other DNA
gcctttcatcaccaccattctgggagggctgtacccatccaagtccatcctcctgtcaggcactgtcctgcccagtgctcagaggttccacatcaacctgtgctctgggaaccacatcgccttccacctgaacccccgttttgatgagaatgctgtggtccgcaacacccagatcgacaactcctgggggtctgaggagcgaagtctgccccgaaaaatgcccttcgtccgtggccagagcttctcagtgtggatcttgtgtgaagctcactgcctcaaggtggccgtggatggtcagcacctgtttgaatactaccatcgcctgaggaacctgcccaccatcaacagactggaagtggggggcgacatccagctgacccatgtgcagacaggaagcggagagggcaggggaagtcttctaacatgcggggacgtggaggaaaatcccggccccatggacaccaccaggtacagcaagtggggcggcagctccgaggaggtccccggagggccctggggacgctgggtgcactggagcaggagacccctcttcttggccctggctgtcctggtcaccacagtcctttgggctgtgattctgagtatcctattgtccaaggcctccacggagcgcgcggcgctgcttgacggccacgacctgctgaggacaaacgcctcgaagcagacggcggcgctgggtgccctgaaggaggaggtcggagact

SEQ ID NO: 13 - DNA, 634 bp, synthetic construct
  source 1..634: mol_type = other DNA
tctctctcagcttcagccactggaaccagggagagcccaatgacgcttgggggcgcgagaactgtgtcatgatgctgcacacggggctgtggaacgacgcaccgtgtgacagcgagaaggacggctggatctgtgagaaaaggcacaactgcggaagcggagccacgaacttctctctgttaaagcaagcaggagatgttgaagaaaaccccgggcctatgaaggcacagacagcactgtctttcttcctcattctcataacatctctgagtggatctcaaggcatattccctttggctttcttcatttatgttcctatgaatgaacaaatcgtcattggaagacttgatgaagatataattctcccttcttcatttgagaggggatccgaagtcgtaatacactggaagtatcaagatagctataaggttcacagttactacaaaggcagtgaccatttggaaagccaagatcccagatatgcaaacaggacatcccttttctataatgagattcaaaatgggaatgcgtcgctatttttcagaagagtaagccttctggacgaaggaatttacacctgctatgtaggaacagcaattcaagtgattacaaacaaagtggtgctaaaggtggg

SEQ ID NO: 14 - DNA, 23 bp, synthetic construct
  source 1..23: mol_type = other DNA
ggtttgtccaaactcatcaatgt

SEQ ID NO: 15 - DNA, 18 bp, synthetic construct
  source 1..18: mol_type = other DNA
ggtgggggttagacccaa

SEQ ID NO: 16 - DNA, 19 bp, synthetic construct
  source 1..19: mol_type = other DNA
gatgttgtgtccctcctgg

SEQ ID NO: 17 - DNA, 24 bp, synthetic construct
  source 1..24: mol_type = other DNA
ggacaaaccacaactagaatgcag

SEQ ID NO: 18 - DNA, 20 bp, synthetic construct
  source 1..20: mol_type = other DNA
accttatattcccagggccg

SEQ ID NO: 19 - DNA, 22 bp, synthetic construct
  source 1..22: mol_type = other DNA
ggctatgaactaatgaccccgt

SEQ ID NO: 20 - DNA, 28 bp, synthetic construct
  source 1..28: mol_type = other DNA
cagctttcttgtacaaagtggggacagg

SEQ ID NO: 21 - DNA, 22 bp, synthetic construct
  source 1..22: mol_type = other DNA
tcccagtgcacccgataatggc

SEQ ID NO: 22 - DNA, 21 bp, synthetic construct
  source 1..21: mol_type = other DNA
tgtcccctccaccccacagtg

SEQ ID NO: 23 - DNA, 6886 bp, synthetic construct
  source 1..6886: mol_type = other DNA
tgctttctctgacctgcattctctcccctgggcctgtgccgctttctgtctgcagcttgtggcctgggtcacctctacggctggcccagatccttccctgccgcctccttcaggttccgtcttcctccactccctcttccccttgctctctgctgtgttgctgcccaaggatgctctttccggagcacttccttctcggcgctgcaccacgtgatgtcctctgagcggatcctccccgtgtctgggtcctctccgggcatctctcctccctcacccaaccccatgccgtcttcactcgctgggttcccttttccttctccttctggggcctgtgccatctctcgtttcttaggatggccttctccgacggatgtctcccttgcgtcccgcctccccttcttgtaggcctgcatcatcaccgtttttctggacaaccccaaagtaccccgtctccctggctttagccacctctccatcctcttgctttctttgcctggacaccccgttctcctgtggattcgggtcacctctcactcctttcatttgggcagctcccctaccccccttacctctctagtctgtgctagctcttccagccccctgtcatggcatcttccaggggtccgagagctcagctagtcttcttcctccaacccgggcccctatgtccacttcaggacagcatgtttgctgcctccagggatcctgtgtccccgagctgggaccaccttatattcccagggccggttaatgtggctctggttctgggtacttttatctgtcccctccaccccacagtggggccactacaagtttgtacaaaaaagcaggctgtcgacattgattattgactagttattaatagtaatcaattacggggtcattagttcatagcccatatatggagttccgcgttacataacttacggtaaatggcccgcctggctgaccgcccaacgacccccgcccattgacgtcaataatgacgtatgttcccatagtaacgccaatagggactttccattgacgtcaatgggtggagtatttacggtaaactgcccacttggcagtacatcaagtgtatcatatgccaagtacgccccctattgacgtcaatgacggtaaatggcccgcctggcattatgcccagtacatgaccttatgggactttcctacttggcagtacatctacgtattagtcatcgctattaccatggtcgaggtgagccccacgttctgcttcactctccccatctcccccccctccccacccccaattttgtatttatttattttttaattattttgtgcagcgatgggggcggggggggggggggggcgcgcgccaggcggggcggggcggggcgaggggcggggcggggcgaggcggagaggtgcggcggcagccaatcagagcggcgcgctccgaaagtttccttttatggcgaggcggcggcggcggcggccctataaaaagcgaagcgcgcggcgggcgggagtcgctgcgcgctgccttcgccccgtgccccgctccgccgccgcctcgcgccgcccgccccggctctgactgaccgcgttactcccacaggtgagcgggcgggacggcccttctcctccgggctgtaattagcgcttggtttaatgacggcttgtttcttttctgtggctgcgtgaaagccttgaggggctccgggagggccctttgtgcggggggagcggctcggggggtgcgtgcgtgtgtgtgtgcgtggggagcgccgcgtgcggctccgcgctgcccggcggctgtgagcgctgcgggcgcggcgcggggctttgtgcgctccgcagtgtgcgcgaggggagcgcggccgggggcggtgccccgcggtgcggggggggctgcgaggggaacaaaggctgcgtgcggggtgtgtgcgtgggggggtgagcagggggtgtgggcgcgtcggtcgggctgcaaccccccctgcacccccctccccgagttgctgagcacggcccggcttcgggtgcggggctccgtacggggcgtggcgcggggctcgccgtgccgggcggggggtggcggcaggtgggggtgccgggcggggcggggccgcctcgggccggggagggctcgggggaggggcgcggcggcccccggagcgccggcggctgtcgaggcgcggcgagccgcagccattgccttttatggtaatcgtgcgagagggcgcagggacttcctttgtcccaaatctgtgcggagccgaaatctgggaggcgccgccgcaccccctctagcgggcgcggggcgaagcggtgcggcgccggcaggaaggaaatgggcggggagggccttcgtgcgtcgccgcgccgccgtccccttctccctctccagcctcggggctgtccgcggggggacggctgccttcgggggggacggggcagggcggggttcggcttctggcgtgtgaccggcggctctagagcctctgctaaccatgttcatgccttcttctttttcctacagctcctgggcaacgtgctggttattgtgctgtctcatcattttggcaaagaattcgccaccatggccttcagcggttcccaggctccctacctgagtccagctgtccccttttctgggactattcaaggaggtctccaggacggacttcagatcactgtcaatgggaccgttctcagctccagtggaaccaggtttgctgtgaactttcagactggcttcagtggaaatgacattgccttccacttcaaccctcggtttgaagatggagggtacgtggtgtgcaacacgaggcagaacggaagctgggggcccgaggagaggaagacacacatgcctttccagaaggggatgccctttgacctctgcttcctggtgcagagctcagatttcaaggtgatggtgaacgggatcctcttcgtgcagtacttccaccgcgtgcccttccaccgtgtggacaccatctccgtcaatggctctgtgcagctgtcctacatcagcttccagaacccccgcacagtccctgttcagcctgccttctccacggtgccgttctcccagcctgtctgtttcccacccaggcccagggggcgcagacaaaaacctcccggcgtgtggcctgccaacccggctcccattacccagacagtcatccacacagtgcagagcgcccctggacagatgttctctactcccgccatcccacctatgatgtacccccaccccgcctatccgatgcctttcatcaccaccattctgggagggctgtacccatccaagtccatcctcctgtcaggcactgtcctgcccagtgctcagaggttccacatcaacctgtgctctgggaaccacatcgccttccacctgaacccccgttttgatgagaatgctgtggtccgcaacacccagatcgacaactcctgggggtctgaggagcgaagtctgccccgaaaaatgcccttcgtccgtggccagagcttctcagtgtggatcttgtgtgaagctcactgcctcaaggtggccgtggatggtcagcacctgtttgaatactaccatcgcctgaggaacctgcccaccatcaacagactggaagtggggggcgacatccagctgacccatgtgcagacaggaagcggagagggcaggggaagtcttctaacatgcggggacgtggaggaaaatcccggccccatggacaccaccaggtacagcaagtggggcggcagctccgaggaggtccccggagggccctggggacgctgggtgcactggagcaggagacccctcttcttggccctggctgtcctggtcaccacagtcctttgggctgtgattctgagtatcctattgtccaaggcctccacggagcgcgcggcgctgcttgacggccacgacctgctgaggacaaacgcctcgaagcagacggcggcgctgggtgccctgaaggaggaggtcggagactgccacagctgctgctcggggacgcaggcgcagctgcagaccacgcgcgcggagcttggggaggcgcaggcgaagctgatggagcaggagagcgccctgcgggaactgcgtgagcgcgtgacccagggcttggctgaagccggcaggggccgtgaggacgtccgcactgagctgttccgggcgctggaggccgtgaggctccagaacaactcctgcgagccgtgccccacgtcgtggctgtccttcgagggctcctgctactttttctctgtgccaaagacgacgtgggcggcggcgcaggatcactgcgcagatgccagcgcgcacctggtgatcgttgggggcctggatgagcagggcttcctcactcggaacacgcgtggccgtggttactggctgggcctgagggctgtgcgccatctgggcaaggttcagggctaccagtgggtggacggagtctctctcagcttcagccactggaaccagggagagcccaatgacgcttgggggcgcgagaactgtgtcatgatgctgcacacggggctgtggaacgacgcaccgtgtgacagcgagaaggacggctggatctgtgagaaaaggcacaactgcggaagcggagccacgaacttctctctgttaaagcaagcaggagatgttgaagaaaaccccgggcctatgaaggcacagacagcactgtctttcttcctcattctcataacatctctgagtggatctcaaggcatattccctttggctttcttcatttatgttcctatgaatgaacaaatcgtcattggaagacttgatgaagatataattctcccttcttcatttgagaggggatccgaagtcgtaatacactggaagtatcaagatagctataaggttcacagttactacaaaggcagtgaccatttggaaagccaagatcccagatatgcaaacaggacatcccttttctataatgagattcaaaatgggaatgcgtcgctatttttcagaagagtaagccttctggacgaaggaatttacacctgctatgtaggaacagcaattcaagtgattacaaacaaagtggtgctaaaggtgggagtttttctcacacccgtgatgaagtatgaaaagaggaacacaaacagcttcttaatatgcagcgtgttaagtgtttatcctcgtccaattatcacgtggaaaatggacaacacacctatctctgaaaacaacatggaagaaacagggtctttggattctttttctattaacagcccactgaatattacaggatcaaattcatcttatgaatgtacaattgaaaattcactgctgaagcaaacatggacagggcgctggacgatgaaagatggccttcataaaatgcaaagtgaacacgtttcactctcatgtcaacctgtaaatgattatttttcaccaaaccaagacttcaaagttacttggtccagaatgaaaagtgggactttctctgtcctggcttactatctgagctcctcacaaaatacaattatcaatgaatcccgattctcatggaacaaagagctgataaaccagagtgacttctctatgaatttgatggatcttaatctttcagacagtggggaatatttatgcaatatttcttcggatgaatatactttacttaccatccacacagtgcatgtagaaccgagccaagaaacagcttcccataacaaaggcttatggattttggtgccctctgcgattttggcagcttttctgctgatttggagcgtaaaatgttgcagagcccagctagaagccaggaggagcagacaccctgctgatggagcccaacaagaaagatgttgtgtccctcctggtgagcgctgtcccagtgcacccgataatggcgaagaaaatgtgcctctttcaggaaaagtatagaacttgtttattgcagcttataatggttacaaataaagcaatagcatcacaaatttcacaaataaagcatttttttcactgcattctagttgtggtttgtccaaactcatcaatgtatcttagtcgacagtactaagcttacccagctttcttgtacaaagtggggacaggattggtgacagaaaagccccatccttaggcctcctccttcctagtctcctgatattgggtctaacccccacctcctgttaggcagattccttatctggtgacacacccccatttcctggagccatctctctccttgccagaacctctaaggtttgcttacgatggagccagagaggatcctgggagggagagcttggcagggggtgggagggaagggggggatgcgtgacctgcccggttctcagtggccaccctgcgctaccctctcccagaacctgagctgctctgacgcggccgtctggtgcgtttcactgatcctggtgctgcagcttccttacacttcccaagaggagaagcagtttggaaaaacaaaatcagaataagttggtcctgagttctaactttggctcttcacctttctagtccccaatttatattgttcctccgtgcgtcagttttacctgtgagataaggccagtagccagccccgtcctggcagggctgtggtgaggaggggggtgtccgtgtggaaaactccctttgtgagaatggtgcgtcctaggtgttcaccaggtcgtggccgcctctactccctttctctttctccatccttctttccttaaagagtccccagtgctatctgggacatattcctccgcccagagcagggtcccgcttccctaaggccctgctctgggcttctgggtttgagtccttggcaagcccaggagaggcgctcaggcttccctgtcccccttcctcgtccaccatctcatgcccctggctctcctgccccttccctacaggggttcctggctctgctct

SEQ ID NO: 24 - DNA, 4636 bp, synthetic construct
  source 1..4636: mol_type = other DNA
tgctttctctgacctgcattctctcccctgggcctgtgccgctttctgtctgcagcttgtggcctgggtcacctctacggctggcccagatccttccctgccgcctccttcaggttccgtcttcctccactccctcttccccttgctctctgctgtgttgctgcccaaggatgctctttccggagcacttccttctcggcgctgcaccacgtgatgtcctctgagcggatcctccccgtgtctgggtcctctccgggcatctctcctccctcacccaaccccatgccgtcttcactcgctgggttcccttttccttctccttctggggcctgtgccatctctcgtttcttaggatggccttctccgacggatgtctcccttgcgtcccgcctccccttcttgtaggcctgcatcatcaccgtttttctggacaaccccaaagtaccccgtctccctggctttagccacctctccatcctcttgctttctttgcctggacaccccgttctcctgtggattcgggtcacctctcactcctttcatttgggcagctcccctaccccccttacctctctagtctgtgctagctcttccagccccctgtcatggcatcttccaggggtccgagagctcagctagtcttcttcctccaacccgggcccctatgtccacttcaggacagcatgtttgctgcctccagggatcctgtgtccccgagctgggaccaccttatattcccagggccggttaatgtggctctggttctgggtacttttatctgtcccctccaccccacagtggggccactacaagtttgtacaaaaaagcaggctgtcgacattgattattgactagttattaatagtaatcaattacggggtcattagttcatagcccatatatggagttccgcgttacataacttacggtaaatggcccgcctggctgaccgcccaacgacccccgcccattgacgtcaataatgacgtatgttcccatagtaacgccaatagggactttccattgacgtcaatgggtggagtatttacggtaaactgcccacttggcagtacatcaagtgtatcatatgccaagtacgccccctattgacgtcaatgacggtaaatggcccgcctggcattatgcccagtacatgaccttatgggactttcctacttggcagtacatctacgtattagtcatcgctattaccatggtcgaggtgagccccacgttctgcttcactctccccatctcccccccctccccacccccaattttgtatttatttattttttaattattttgtgcagcgatgggggcggggggggggggggggcgcgcgccaggcggggcggggcggggcgaggggcggggcggggcgaggcggagaggtgcggcggcagccaatcagagcggcgcgctccgaaagtttccttttatggcgaggcggcggcggcggcggccctataaaaagcgaagcgcgcggcgggcgggagtcgctgcgcgctgccttcgccccgtgccccgctccgccgccgcctcgcgccgcccgccccggctctgactgaccgcgttactcccacaggtgagcgggcgggacggcccttctcctccgggctgtaattagcgcttggtttaatgacggcttgtttcttttctgtggctgcgtgaaagccttgaggggctccgggagggccctttgtgcggggggagcggctcggggggtgcgtgcgtgtgtgtgtgcgtggggagcgccgcgtgcggctccgcgctgcccggcggctgtgagcgctgcgggcgcggcgcggggctttgtgcgctccgcagtgtgcgcgaggggagcgcggccgggggcggtgccccgcggtgcggggggggctgcgaggggaacaaaggctgcgtgcggggtgtgtgcgtgggggggtgagcagggggtgtgggcgcgtcggtcgggctgcaaccccccctgcacccccctccccgagttgctgagcacggcccggcttcgggtgcggggctccgtacggggcgtggcgcggggctcgccgtgccgggcggggggtggcggcaggtgggggtgccgggcggggcggggccgcctcgggccggggagggctcgggggaggggcgcggcggcccccggagcgccggcggctgtcgaggcgcggcgagccgcagccattgccttttatggtaatcgtgcgagagggcgcagggacttcctttgtcccaaatctgtgcggagccgaaatctgggaggcgccgccgcaccccctctagcgggcgcggggcgaagcggtgcggcgccggcaggaaggaaatgggcggggagggccttcgtgcgtcgccgcgccgccgtccccttctccctctccagcctcggggctgtccgcggggggacggctgccttcgggggggacggggcagggcggggttcggcttctggcgtgtgaccggcggctctagagcctctgctaaccatgttcatgccttcttctttttcctacagctcctgggcaacgtgctggttattgtgctgtctcatcattttggcaaagaattcgccaccatggccttcagcggttcccaggctccctacctgagtccagctgtccccttttctgggactattcaaggaggtctccaggacggacttcagatcactgtcaatgggaccgttctcagctccagtggaaccaggtttgctgtgaactttcagactggcttcagtggaaatgacattgccttccacttcaaccctcggtttgaagatggagggtacgtggtgtgcaacacgaggcagaacggaagctgggggcccgaggagaggaagacacacatgcctttccagaaggggatgccctttgacctctgcttcctggtgcagagctcagatttcaaggtgatggtgaacgggatcctcttcgtgcagtacttccaccgcgtgcccttccaccgtgtggacaccatctccgtcaatggctctgtgcagctgtcctacatcagcttccagaacccccgcacagtccctgttcagcctgccttctccacggtgccgttctcccagcctgtctgtttcccacccaggcccagggggcgcagacaaaaacctcccggcgtgtggcctgccaacccggctcccattacccagacagtcatccacacagtgcagagcgcccctggacagatgttctctactcccgccatcccacctatgatgtacccccaccccgcctatccgatgcctttcatcaccaccattctgggagggctgtacccatccaagtccatcctcctgtcaggcactgtcctgcccagtgctcagaggttccacatcaacctgtgctctgggaaccacatcgccttccacctgaacccccgttttgatgagaatgctgtggtccgcaacacccagatcgacaactcctgggggtctgaggagcgaagtctgccccgaaaaatgcccttcgtccgtggccagagcttctcagtgtggatcttgtgtgaagctcactgcctcaaggtggccgtggatggtcagcacctgtttgaatactaccatcgcctgaggaacctgcccaccatcaacagactggaagtggggggcgacatccagctgacccatgtgcagacatagaacttgtttattgcagcttataatggttacaaataaagcaatagcatcacaaatttcacaaataaagcatttttttcactgcattctagttgtggtttgtccaaactcatcaatgtatcttagtcgacagtactaagcttacccagctttcttgtacaaagtggggacaggattggtgacagaaaagccccatccttaggcctcctccttcctagtctcctgatattgggtctaacccccacctcctgttaggcagattccttatctggtgacacacccccatttcctggagccatctctctccttgccagaacctctaaggtttgcttacgatggagccagagaggatcctgggagggagagcttggcagggggtgggagggaagggggggatgcgtgacctgcccggttctcagtggccaccctgcgctaccctctcccagaacctgagctgctctgacgcggccgtctggtgcgtttcactgatcctggtgctgcagcttccttacacttcccaagaggagaagcagtttggaaaaacaaaatcagaataagttggtcctgagttctaactttggctcttcacctttctagtccccaatttatattgttcctccgtgcgtcagttttacctgtgagataaggccagtagccagccccgtcctggcagggctgtggtgaggaggggggtgtccgtgtggaaaactccctttgtgagaatggtgcgtcctaggtgttcaccaggtcgtggccgcctctactccctttctctttctccatccttctttccttaaagagtccccagtgctatctgggacatattcctccgcccagagcagggtcccgcttccctaaggccctgctctgggcttctgggtttgagtccttggcaagcccaggagaggcgctcaggcttccctgtcccccttcctcgtccaccatctcatgcccctggctctcctgccccttccctacaggggttcctggctctgctct

SEQ ID NO: 25 - DNA, 4450 bp, synthetic construct
  source 1..4450: mol_type = other DNA
tgctttctctgacctgcattctctcccctgggcctgtgccgctttctgtctgcagcttgtggcctgggtcacctctacggctggcccagatccttccctgccgcctccttcaggttccgtcttcctccactccctcttccccttgctctctgctgtgttgctgcccaaggatgctctttccggagcacttccttctcggcgctgcaccacgtgatgtcctctgagcggatcctccccgtgtctgggtcctctccgggcatctctcctccctcacccaaccccatgccgtcttcactcgctgggttcccttttccttctccttctggggcctgtgccatctctcgtttcttaggatggccttctccgacggatgtctcccttgcgtcccgcctccccttcttgtaggcctgcatcatcaccgtttttctggacaaccccaaagtaccccgtctccctggctttagccacctctccatcctcttgctttctttgcctggacaccccgttctcctgtggattcgggtcacctctcactcctttcatttgggcagctcccctaccccccttacctctctagtctgtgctagctcttccagccccctgtcatggcatcttccaggggtccgagagctcagctagtcttcttcctccaacccgggcccctatgtccacttcaggacagcatgtttgctgcctccagggatcctgtgtccccgagctgggaccaccttatattcccagggccggttaatgtggctctggttctgggtacttttatctgtcccctccaccccacagtggggccactacaagtttgtacaaaaaagcaggctgtcgacattgattattgactagttattaatagtaatcaattacggggtcattagttcatagcccatatatggagttccgcgttacataacttacggtaaatggcccgcctggctgaccgcccaacgacccccgcccattgacgtcaataatgacgtatgttcccatagtaacgccaatagggactttccattgacgtcaatgggtggagtatttacggtaaactgcccacttggcagtacatcaagtgtatcatatgccaagtacgccccctattgacgtcaatgacggtaaatggcccgcctggcattatgcccagtacatgaccttatgggactttcctacttggcagtacatctacgtattagtcatcgctattaccatggtcgaggtgagccccacgttctgcttcactctccccatctcccccccctccccacccccaattttgtatttatttattttttaattattttgtgcagcgatgggggcggggggggggggggggcgcgcgccaggcggggcggggcggggcgaggggcggggcggggcgaggcggagaggtgcggcggcagccaatcagagcggcgcgctccgaaagtttccttttatggcgaggcggcggcggcggcggccctataaaaagcgaagcgcgcggcgggcgggagtcgctgcgcgctgccttcgccccgtgccccgctccgccgccgcctcgcgccgcccgccccggctctgactgaccgcgttactcccacaggtgagcgggcgggacggcccttctcctccgggctgtaattagcgcttggtttaatgacggcttgtttcttttctgtggctgcgtgaaagccttgaggggctccgggagggccctttgtgcggggggagcggctcggggggtgcgtgcgtgtgtgtgtgcgtggggagcgccgcgtgcggctccgcgctgcccggcggctgtgagcgctgcgggcgcggcgcggggctttgtgcgctccgcagtgtgcgcgaggggagcgcggccgggggcggtgccccgcggtgcggggggggctgcgaggggaacaaaggctgcgtgcggggtgtgtgcgtgggggggtgagcagggggtgtgggcgcgtcggtcgggctgcaaccccccctgcacccccctccccgagttgctgagcacggcccggcttcgggtgcggggctccgtacggggcgtggcgcggggctcgccgtgccgggcggggggtggcggcaggtgggggtgccgggcggggcggggccgcctcgggccggggagggctcgggggaggggcgcggcggcccccggagcgccggcggctgtcgaggcgcggcgagccgcagccattgccttttatggtaatcgtgcgagagggcgcagggacttcctttgtcccaaatctgtgcggagccgaaatctgggaggcgccgccgcaccccctctagcgggcgcggggcgaagcggtgcggcgccggcaggaaggaaatgggcggggagggccttcgtgcgtcgccgcgccgccgtccccttctccctctccagcctcggggctgtccgcggggggacggctgccttcgggggggacggggcagggcggggttcggcttctggcgtgtgaccggcggctctagagcctctgctaaccatgttcatgccttcttctttttcctacagctcctgggcaacgtgctggttattgtgctgtctcatcattttggcaaagaattcgccaccatggacaccaccaggtacagcaagtggggcggcagctccgaggaggtccccggagggccctggggacgctgggtgcactggagcaggagacccctcttcttggccctggctgtcctggtcaccacagtcctttgggctgtgattctgagtatcctattgtccaaggcctccacggagcgcgcggcgctgcttgacggccacgacctgctgaggacaaacgcctcgaagcagacggcggcgctgggtgccctgaaggaggaggtcggagactgccacagctgctgctcggggacgcaggcgcagctgcagaccacgcgcgcggagcttggggaggcgcaggcgaagctgatggagcaggagagcgccctgcgggaactgcgtgagcgcgtgacccagggcttggctgaagccggcaggggccgtgaggacgtccgcactgagctgttccgggcgctggaggccgtgaggctccagaacaactcctgcgagccgtgccccacgtcgtggctgtccttcgagggctcctgctactttttctctgtgccaaagacgacgtgggcggcggcgcaggatcactgcgcagatgccagcgcgcacctggtgatcgttgggggcctggatgagcagggcttcctcactcggaacacgcgtggccgtggttactggctgggcctgagggctgtgcgccatctgggcaaggttcagggctaccagtgggtggacggagtctctctcagcttcagccactggaaccagggagagcccaatgacgcttgggggcgcgagaactgtgtcatgatgctgcacacggggctgtggaacgacgcaccgtgtgacagcgagaaggacggctggatctgtgagaaaaggcacaactgctagaacttgtttattgcagcttataatggttacaaataaagcaatagcatcacaaatttcacaaataaagcatttttttcactgcattctagttgtggtttgtccaaactcatcaatgtatcttagtcgacagtactaagcttacccagctttcttgtacaaagtggggacaggattggtgacagaaaagccccatccttaggcctcctccttcctagtctcctgatattgggtctaacccccacctcctgttaggcagattccttatctggtgacacacccccatttcctggagccatctctctccttgccagaacctctaaggtttgcttacgatggagccagagaggatcctgggagggagagcttggcagggggtgggagggaagggggggatgcgtgacctgcccggttctcagtggccaccctgcgctaccctctcccagaacctgagctgctctgacgcggccgtctggtgcgtttcactgatcctggtgctgcagcttccttacacttcccaagaggagaagcagtttggaaaaacaaaatcagaataagttggtcctgagttctaactttggctcttcacctttctagtccccaatttatattgttcctccgtgcgtcagttttacctgtgagataaggccagtagccagccccgtcctggcagggctgtggtgaggaggggggtgtccgtgtggaaaactccctttgtgagaatggtgcgtcctaggtgttcaccaggtcgtggccgcctctactccctttctctttctccatccttctttccttaaagagtccccagtgctatctgggacatattcctccgcccagagcagggtcccgcttccctaaggccctgctctgggcttctgggtttgagtccttggcaagcccaggagaggcgctcaggcttccctgtcccccttcctcgtccaccatctcatgcccctggctctcctgccccttccctacaggggttcctggctctgctct

SEQ ID NO: 26 - DNA, 5578 bp, synthetic construct
  source 1..5578: mol_type = other DNA
tgctttctctgacctgcattctctcccctgggcctgtgccgctttctgtctgcagcttgtggcctgggtcacctctacggctggcccagatccttccctgccgcctccttcaggttccgtcttcctccactccctcttccccttgctctctgctgtgttgctgcccaaggatgctctttccggagcacttccttctcggcgctgcaccacgtgatgtcctctgagcggatcctccccgtgtctgggtcctctccgggcatctctcctccctcacccaaccccatgccgtcttcactcgctgggttcccttttccttctccttctggggcctgtgccatctctcgtttcttaggatggccttctccgacggatgtctcccttgcgtcccgcctccccttcttgtaggcctgcatcatcaccgtttttctggacaaccccaaagtaccccgtctccctggctttagccacctctccatcctcttgctttctttgcctggacaccccgttctcctgtggattcgggtcacctctcactcctttcatttgggcagctcccctaccccccttacctctctagtctgtgctagctcttccagccccctgtcatggcatcttccaggggtccgagagctcagctagtcttcttcctccaacccgggcccctatgtccacttcaggacagcatgtttgctgcctccagggatcctgtgtccccgagctgggaccaccttatattcccagggccggttaatgtggctctggttctgggtacttttatctgtcccctccaccccacagtggggccactacaagtttgtacaaaaaagcaggctgtcgacattgattattgactagttattaatagtaatcaattacggggtcattagttcatagcccatatatggagttccgcgttacataacttacggtaaatggcccgcctggctgaccgcccaacgacccccgcccattgacgtcaataatgacgtatgttcccatagtaacgccaatagggactttccattgacgtcaatgggtggagtatttacggtaaactgcccacttggcagtacatcaagtgtatcatatgccaagtacgccccctattgacgtcaatgacggtaaatggcccgcctggcattatgcccagtacatgaccttatgggactttcctacttggcagtacatctacgtattagtcatcgctattaccatggtcgaggtgagccccacgttctgcttcactctccccatctcccccccctccccacccccaattttgtatttatttattttttaattattttgtgcagcgatgggggcggggggggggggggggcgcgcgccaggcggggcggggcggggcgaggggcggggcggggcgaggcggagaggtgcggcggcagccaatcagagcggcgcgctccgaaagtttccttttatggcgaggcggcggcggcggcggccctataaaaagcgaagcgcgcggcgggcgggagtcgctgcgcgctgccttcgccccgtgccccgctccgccgccgcctcgcgccgcccgccccggctctgactgaccgcgttactcccacaggtgagcgggcgggacggcccttctcctccgggctgtaattagcgcttggtttaatgacggcttgtttcttttctgtggctgcgtgaaagccttgaggggctccgggagggccctttgtgcggggggagcggctcggggggtgcgtgcgtgtgtgtgtgcgtggggagcgccgcgtgcggctccgcgctgcccggcggctgtgagcgctgcgggcgcggcgcggggctttgtgcgctccgcagtgtgcgcgaggggagcgcggccgggggcggtgccccgcggtgcggggggggctgcgaggggaacaaaggctgcgtgcggggtgtgtgcgtgggggggtgagcagggggtgtgggcgcgtcggtcgggctgcaaccccccctgcacccccctccccgagttgctgagcacggcccggcttcgggtgcggggctccgtacggggcgtggcgcggggctcgccgtgccgggcggggggtggcggcaggtgggggtgccgggcggggcggggccgcctcgggccggggagggctcgggggaggggcgcggcggcccccggagcgccggcggctgtcgaggcgcggcgagccgcagccattgccttttatggtaatcgtgcgagagggcgcagggacttcctttgtcccaaatctgtgcggagccgaaatctgggaggcgccgccgcaccccctctagcgggcgcggggcgaagcggtgcggcgccggcaggaaggaaatgggcggggagggccttcgtgcgtcgccgcgccgccgtccccttctccctctccagcctcggggctgtccgcggggggacggctgccttcgggggggacggggcagggcggggttcggcttctggcgtgtgaccggcggctctagagcctctgctaaccatgttcatgccttcttctttttcctacagctcctgggcaacgtgctggttattgtgctgtctcatcattttggcaaagaattcgccaccatggccttcagcggttcccaggctccctacctgagtccagctgtccccttttctgggactattcaaggaggtctccaggacggacttcagatcactgtcaatgggaccgttctcagctccagtggaaccaggtttgctgtgaactttcagactggcttcagtggaaatgacattgccttccacttcaaccctcggtttgaagatggagggtacgtggtgtgcaacacgaggcagaacggaagctgggggcccgaggagaggaagacacacatgcctttccagaaggggatgccctttgacctctgcttcctggtgcagagctcagatttcaaggtgatggtgaacgggatcctcttcgtgcagtacttccaccgcgtgcccttccaccgtgtggacaccatctccgtcaatggctctgtgcagctgtcctacatcagcttccagaacccccgcacagtccctgttcagcctgccttctccacggtgccgttctcccagcctgtctgtttcccacccaggcccagggggcgcagacaaaaacctcccggcgtgtggcctgccaacccggctcccattacccagacagtcatccacacagtgcagagcgcccctggacagatgttctctactcccgccatcccacctatgatgtacccccaccccgcctatccgatgcctttcatcaccaccattctgggagggctgtacccatccaagtccatcctcctgtcaggcactgtcctgcccagtgctcagaggttccacatcaacctgtgctctgggaaccacatcgccttccacctgaacccccgttttgatgagaatgctgtggtccgcaacacccagatcgacaactcctgggggtctgaggagcgaagtctgccccgaaaaatgcccttcgtccgtggccagagcttctcagtgtggatcttgtgtgaagctcactgcctcaaggtggccgtggatggtcagcacctgtttgaatactaccatcgcctgaggaacctgcccaccatcaacagactggaagtggggggcgacatccagctgacccatgtgcagacaggaagcggagagggcaggggaagtcttctaacatgcggggacgtggaggaaaatcccggccccatggacaccaccaggtacagcaagtggggcggcagctccgaggaggtccccggagggccctggggacgctgggtgcactggagcaggagacccctcttcttggccctggctgtcctggtcaccacagtcctttgggctgtgattctgagtatcctattgtccaaggcctccacggagcgcgcggcgctgcttgacggccacgacctgctgaggacaaacgcctcgaagcagacggcggcgctgggtgccctgaaggaggaggtcggagactgccacagctgctgctcggggacgcaggcgcagctgcagaccacgcgcgcggagcttggggaggcgcaggcgaagctgatggagcaggagagcgccctgcgggaactgcgtgagcgcgtgacccagggcttggctgaagccggcaggggccgtgaggacgtccgcactgagctgttccgggcgctggaggccgtgaggctccagaacaactcctgcgagccgtgccccacgtcgtggctgtccttcgagggctcctgctactttttctctgtgccaaagacgacgtgggcggcggcgcaggatcactgcgcagatgccagcgcgcacctggtgatcgttgggggcctggatgagcagggcttcctcactcggaacacgcgtggccgtggttactggctgggcctgagggctgtgcgccatctgggcaaggttcagggctaccagtgggtggacggagtctctctcagcttcagccactggaaccagggagagcccaatgacgcttgggggcgcgagaactgtgtcatgatgctgcacacggggctgtggaacgacgcaccgtgtgacagcgagaaggacggctggatctgtgagaaaaggcacaactgctagaacttgtttattgcagcttataatggttacaaataaagcaatagcatcacaaatttcacaaataaagcatttttttcactgcattctagttgtggtttgtccaaactcatcaatgtatcttagtcgacagtactaagcttacccagctttcttgtacaaagtggggacaggattggtgacagaaaagccccatccttaggcctcctccttcctagtctcctgatattgggtctaacccccacctcctgttaggcagattccttatctggtgacacacccccatttcctggagccatctctctccttgccagaacctctaaggtttgcttacgatggagccagagaggatcctgggagggagagcttggcagggggtgggagggaagggggggatgcgtgacctgcccggttctcagtggccaccctgcgctaccctctcccagaacctgagctgctctgacgcggccgtctggtgcgtttcactgatcctggtgctgcagcttccttacacttcccaagaggagaagcagtttggaaaaacaaaatcagaataagttggtcctgagttctaactttggctcttcacctttctagtccccaatttatattgttcctccgtgcgtcagttttacctgtgagataaggccagtagccagccccgtcctggcagggctgtggtgaggaggggggtgtccgtgtggaaaactccctttgtgagaatggtgcgtcctaggtgttcaccaggtcgtggccgcctctactccctttctctttctccatccttctttccttaaagagtccccagtgctatctgggacatattcctccgcccagagcagggtcccgcttccctaaggccctgctctgggcttctgggtttgagtccttggcaagcccaggagaggcgctcaggcttccctgtcccccttcctcgtccaccatctcatgcccctggctctcctgccccttccctacaggggttcctggctctgctct

SEQ ID NO: 27 - DNA, 6522 bp, synthetic construct
  source 1..6522: mol_type = other DNA
gcattctctcccctgggcctgtgccgctttctgtctgcagcttgtggcctgggtcacctctacggctggcccagatccttccctgccgcctccttcaggttccgtcttcctccactccctcttccccttgctctctgctgtgttgctgcccaaggatgctctttccggagcacttccttctcggcgctgcaccacgtgatgtcctctgagcggatcctccccgtgtctgggtcctctccgggcatctctcctccctcacccaaccccatgccgtcttcactcgctgggttcccttttccttctccttctggggcctgtgccatctctcgtttcttaggatggccttctccgacggatgtctcccttgcgtcccgcctccccttcttgtaggcctgcatcatcaccgtttttctggacaaccccaaagtaccccgtctccctggctttagccacctctccatcctcttgctttctttgcctggacaccccgttctcctgtggattcgggtcacctctcactcctttcatttgggcagctcccctaccccccttacctctctagtctgtgctagctcttccagccccctgtcatggcatcttccaggggtccgagagctcagctagtcttcttcctccaacccgggcccctatgtccacttcaggacagcatgtttgctgcctccagggatcctgtgtccccgagctgggaccaccttatattcccagggccggttaatgtggctctggttctgggtacttttatctgtcccctccaccccacagtggggcaagtttgtacaaaaaagcaggctgtcgacattgattattgactagttattaatagtaatcaattacggggtcattagttcatagcccatatatggagttccgcgttacataacttacggtaaatggcccgcctggctgaccgcccaacgacccccgcccattgacgtcaataatgacgtatgttcccatagtaacgccaatagggactttccattgacgtcaatgggtggagtatttacggtaaactgcccacttggcagtacatcaagtgtatcatatgccaagtacgccccctattgacgtcaatgacggtaaatggcccgcctggcattatgcccagtacatgaccttatgggactttcctacttggcagtacatctacgtattagtcatcgctattaccatggtcgaggtgagccccacgttctgcttcactctccccatctcccccccctccccacccccaattttgtatttatttattttttaattattttgtgcagcgatgggggcggggggggggggggggcgcgcgccaggcggggcggggcggggcgaggggcggggcggggcgaggcggagaggtgcggcggcagccaatcagagcggcgcgctccgaaagtttccttttatggcgaggcggcggcggcggcggccctataaaaagcgaagcgcgcggcgggcgggagtcgctgcgcgctgccttcgccccgtgccccgctccgccgccgcctcgcgccgcccgccccggctctgactgaccgcgttactcccacaggtgagcgggcgggacggcccttctcctccgggctgtaattagcgcttggtttaatgacggcttgtttcttttctgtggctgcgtgaaagccttgaggggctccgggagggccctttgtgcggggggagcggctcggggggtgcgtgcgtgtgtgtgtgcgtggggagcgccgcgtgcggctccgcgctgcccggcggctgtgagcgctgcgggcgcggcgcggggctttgtgcgctccgcagtgtgcgcgaggggagcgcggccgggggcggtgccccgcggtgcggggggggctgcgaggggaacaaaggctgcgtgcggggtgtgtgcgtgggggggtgagcagggggtgtgggcgcgtcggtcgggctgcaaccccccctgcacccccctccccgagttgctgagcacggcccggcttcgggtgcggggctccgtacggggcgtggcgcggggctcgccgtgccgggcggggggtggcggcaggtgggggtgccgggcggggcggggccgcctcgggccggggagggctcgggggaggggcgcggcggcccccggagcgccggcggctgtcgaggcgcggcgagccgcagccattgccttttatggtaatcgtgcgagagggcgcagggacttcctttgtcccaaatctgtgcggagccgaaatctgggaggcgccgccgcaccccctctagcgggcgcggggcgaagcggtgcggcgccggcaggaaggaaatgggcggggagggccttcgtgcgtcgccgcgccgccgtccccttctccctctccagcctcggggctgtccgcggggggacggctgccttcgggggggacggggcagggcggggttcggcttctggcgtgtgaccggcggctctagagcctctgctaaccatgttcatgccttcttctttttcctacagctcctgggcaacgtgctggttattgtgctgtctcatcattttggcaaagaattcacccagctttcttgtacaaagtgggccaccatggccttcagcggttcccaggctccctacctgagtccagctgtccccttttctgggactattcaaggaggtctccaggacggacttcagatcactgtcaatgggaccgttctcagctccagtggaaccaggtttgctgtgaactttcagactggcttcagtggaaatgacattgccttccacttcaaccctcggtttgaagatggagggtacgtggtgtgcaacacgaggcagaacggaagctgggggcccgaggagaggaagacacacatgcctttccagaaggggatgccctttgacctctgcttcctggtgcagagctcagatttcaaggtgatggtgaacgggatcctcttcgtgcagtacttccaccgcgtgcccttccaccgtgtggacaccatctccgtcaatggctctgtgcagctgtcctacatcagcttccagaacccccgcacagtccctgttcagcctgccttctccacggtgccgttctcccagcctgtctgtttcccacccaggcccagggggcgcagacaaaaacctcccggcgtgtggcctgccaacccggctcccattacccagacagtcatccacacagtgcagagcgcccctggacagatgttctctactcccgccatcccacctatgatgtacccccaccccgcctatccgatgcctttcatcaccaccattctgggagggctgtacccatccaagtccatcctcctgtcaggcactgtcctgcccagtgctcagaggttccacatcaacctgtgctctgggaaccacatcgccttccacctgaacccccgttttgatgagaatgctgtggtccgcaacacccagatcgacaactcctgggggtctgaggagcgaagtctgccccgaaaaatgcccttcgtccgtggccagagcttctcagtgtggatcttgtgtgaagctcactgcctcaaggtggccgtggatggtcagcacctgtttgaatactaccatcgcctgaggaacctgcccaccatcaacagactggaagtggggggcgacatccagctgacccatgtgcagacaggaagcggagagggcaggggaagtcttctaacatgcggggacgtggaggaaaatcccggccccatggacaccaccaggtacagcaagtggggcggcagctccgaggaggtccccggagggccctggggacgctgggtgcactggagcaggagacccctcttcttggccctggctgtcctggtcaccacagtcctttgggctgtgattctgagtatcctattgtccaaggcctccacggagcgcgcggcgctgcttgacggccacgacctgctgaggacaaacgcctcgaagcagacggcggcgctgggtgccctgaaggaggaggtcggagactgccacagctgctgctcggggacgcaggcgcagctgcagaccacgcgcgcggagcttggggaggcgcaggcgaagctgatggagcaggagagcgccctgcgggaactgcgtgagcgcgtgacccagggcttggctgaagccggcaggggccgtgaggacgtccgcactgagctgttccgggcgctggaggccgtgaggctccagaacaactcctgcgagccgtgccccacgtcgtggctgtccttcgagggctcctgctactttttctctgtgccaaagacgacgtgggcggcggcgcaggatcactgcgcagatgccagcgcgcacctggtgatcgttgggggcctggatgagcagggcttcctcactcggaacacgcgtggccgtggttactggctgggcctgagggctgtgcgccatctgggcaaggttcagggctaccagtgggtggacggagtctctctcagcttcagccactggaaccagggagagcccaatgacgcttgggggcgcgagaactgtgtcatgatgctgcacacggggctgtggaacgacgcaccgtgtgacagcgagaaggacggctggatctgtgagaaaaggcacaactgcggaagcggagccacgaacttctctctgttaaagcaagcaggagatgttgaagaaaaccccgggcctatgaggatatttgctgtctttatattcatgacctactggcatttgctgaacgcatttactgtcacggttcccaaggacctatatgtggtagagtatggtagcaatatgacaattgaatgcaaattcccagtagaaaaacaattagacctggctgcactaattgtctattgggaaatggaggataagaacattattcaatttgtgcatggagaggaagacctgaaggttcagcatagtagctacagacagagggcccggctgttgaaggaccagctctccctgggaaatgctgcacttcagatcacagatgtgaaattgcaggatgcaggggtgtaccgctgcatgatcagctatggtggtgccgactacaagcgaattactgtgaaagtcaatgccccatacaacaaaatcaaccaaagaattttggttgtggatccagtcacctctgaacatgaactgacatgtcaggctgagggctaccccaaggccgaagtcatctggacaagcagtgaccatcaagtcctgagtggtaagaccaccaccaccaattccaagagagaggagaagcttttcaatgtgaccagcacactgagaatcaacacaacaactaatgagattttctactgcacttttaggagattagatcctgaggaaaaccatacagctgaattggtcatcccagaactacctctggcacatcctccaaatgaaaggactcacttggtaattctgggagccatcttattatgccttggtgtagcactgacattcatcttccgtttaagaaaagggagaatgatggatgtgaaaaaatgtggcatccaagatacaaactcaaagaagcaaagtgatacacatttggaggagacgtaatagaacttgtttattgcagcttataatggttacaaataaagcaatagcatcacaaatttcacaaataaagcatttttttcactgcattctagttgtggtttgtccaaactcatcaatgtatcttagtcgacagtactaagcttacccagctttcttgtacaaagtggagggacaggattggtgacagaaaagccccatccttaggcctcctccttcctagtctcctgatattgggtctaacccccacctcctgttaggcagattccttatctggtgacacacccccatttcctggagccatctctctccttgccagaacctctaaggtttgcttacgatggagccagagaggatcctgggagggagagcttggcagggggtgggagggaagggggggatgcgtgacctgcccggttctcagtggccaccctgcgctaccctctcccagaacctgagctgctctgacgcggccgtctggtgcgtttcactgatcctggtgctgcagcttccttacacttcccaagaggagaagcagtttggaaaaacaaaatcagaataagttggtcctgagttctaactttggctcttcacctttctagtccccaatttatattgttcctccgtgcgtcagttttacctgtgagataaggccagtagccagccccgtcctggcagggctgtggtgaggaggggggtgtccgtgtggaaaactccctttgtgagaatggtgcgtcctaggtgttcaccaggtcgtggccgcctctactccctttctctttctccatccttctttccttaaagagtccccagtgctatctgggacatattcctccgcccagagcagggtcccgcttccctaaggccctgctctgggcttctgggtttgagtccttggcaagcccaggagaggcgctcaggcttccctgtcccccttcctcgtccaccatctcatgcccctggctctcctgccccttccctacaggggttcctggctctgctct